European Patent Specification EP 3 793 580 B1, published July 31, 2024. Title: Probiotic Lactobacillus kefiri SGL 13 strain and its use for the prevention and the treatment of intestinal inflammation and in the prevention of intestinal cancer. Applicant: SINTAL DIETETICS S.R.L. The sequence listing filed with the application follows.

SEQUENCE LISTING (4 sequences)

SEQ ID NO: 1 - DNA, 20 bp, Artificial Sequence
  16S-27 For Primer
agagtttgatcctggctcag

SEQ ID NO: 2 - DNA, 19 bp, Artificial Sequence
  16-1552 Rev Primer
aaggaggtgwtcarccgca

SEQ ID NO: 3 - DNA, 21 bp, Artificial Sequence
  Lk1 Primer
caacaatcaaaggggttgttg

SEQ ID NO: 4 - DNA, 21 bp, Artificial Sequence
  Lk2 Primer
tcactaggagtaattgaacca